European Patent Application EP 4 299 590 A1, published January 3, 2024. Title: Anti-Siglec15 antibody and use thereof. Applicant: CSPC MEGALITH BIOPHARMACEUTICAL CO., LTD. The sequence listing filed with the application follows.

SEQUENCE LISTING (33 sequences)

SEQ ID NO: 1 - protein, 328 aa, Homo sapiens
MGLSITLLACLATVLPTGSFVATLIATTGALLATGVHSSPAGATSMGVPPGVSAGAGAAAVLPCTPTHPHAHTAGPLTAITAAGGPTAGPGVPACAAAAGSGLCGTALSLHGAPALLGAPAAAALSLAVGALALAAAAATPCAVGPAGAVHAATGSAHGVALHVTAAPAIVAISVLPSPAHAPAALCTAGGGPPPALATSGPALGASLAAVASPAGGHGHLVTAGLPALTHAGATTCTAAASLGASGASVTLPAPHGASGASTVALLLGALGPLALLLLGVLAAAAAAAAPGHLATPATPPASGAGGSATGALSGMAPASPPATMCSP

SEQ ID NO: 2 - protein, 494 aa, Artificial Sequence
  The amino acid sequence of Siglec15-ECD-Fc
MEKSIWLLACLAWVLPTGSFVRTKIDTTENLLNTEVHSSPAQRWSMQVPPEVSAEAGDAAVLPCTFTHPHRHYDGPLTAIWRAGEPYAGPQVFRCAAARGSELCQTALSLHGRFRLLGNPRRNDLSLRVERLALADDRRYFCRVEFAGDVHDRYESRHGVRLHVTAAPRIVNISVLPSPAHAFRALCTAEGEPPPALAWSGPALGNSLAAVRSPREGHGHLVTAELPALTHDGRYTCTAANSLGRSEASVYLFRFHGASGASTPKSCDKTHTCPPCPAPELLGGPSVFLFPPKPKDTLMISRTPEVTCVVVDVSHEDPEVKFNWYVDGVEVHNAKTKPREEQYNSTYRVVSVLTVLHQDWLNGKEYKCKVSNKALPAPIEKTISKAKGQPREPQVYTLPPSRDELTKNQVSLTCLVKGFYPSDIAVEWESNGQPENNYKTTPPVLDSDGSFFLYSKLTVDKSRWQQGNVFSCSVMHEALHNHYTQKSLSLSPGK

SEQ ID NO: 3 - protein, 396 aa, Artificial Sequence
  The amino acid sequence of Siglec15-IgV-Fc
MEKSIWLLACLAWVLPTGSFVRTKIDTTENLLNTEVHSSPAQRWSMQVPPEVSAEAGDAAVLPCTFTHPHRHYDGPLTAIWRAGEPYAGPQVFRCAAARGSELCQTALSLHGRFRLLGNPRRNDLSLRVERLALADDRRYFCRVEFAGDVHDRYESRHGVRLHVTPKSCDKTHTCPPCPAPELLGGPSVFLFPPKPKDTLMISRTPEVTCVVVDVSHEDPEVKFNWYVDGVEVHNAKTKPREEQYNSTYRVVSVLTVLHQDWLNGKEYKCKVSNKALPAPIEKTISKAKGQPREPQVYTLPPSRDELTKNQVSLTCLVKGFYPSDIAVEWESNGQPENNYKTTPPVLDSDGSFFLYSKLTVDKSRWQQGNVFSCSVMHEALHNHYTQKSLSLSPGK

SEQ ID NO: 4 - protein, 270 aa, Artificial Sequence
  The amino acid sequence of Siglec15-ECD-His
MEKSIWLLACLAWVLPTGSFVRTKIDTTENLLNTEVHSSPAQRWSMQVPPEVSAEAGDAAVLPCTFTHPHRHYDGPLTAIWRAGEPYAGPQVFRCAAARGSELCQTALSLHGRFRLLGNPRRNDLSLRVERLALADDRRYFCRVEFAGDVHDRYESRHGVRLHVTAAPRIVNISVLPSPAHAFRALCTAEGEPPPALAWSGPALGNSLAAVRSPREGHGHLVTAELPALTHDGRYTCTAANSLGRSEASVYLFRFHGASGASTHHHHHHH

SEQ ID NO: 5 - protein, 640 aa, Homo sapiens
MLNKMTLHPQQIMIGPRFNRALFDPLLVVLLALQLLVVAGLVRAQTCPSVCSCSNQFSKVICVRKNLREVPDGISTNTRLLNLHENQIQIIKVNSFKHLRHLEILQLSRNHIRTIEIGAFNGLANLNTLELFDNRLTTIPNGAFVYLSKLKELWLRNNPIESIPSYAFNRIPSLRRLDLGELKRLSYISEGAFEGLSNLRYLNLAMCNLREIPNLTPLIKLDELDLSGNHLSAIRPGSFQGLMHLQKLWMIQSQIQVIERNAFDNLQSLVEINLAHNNLTLLPHDLFTPLHHLERIHLHHNPWNCNCDILWLSWWIKDMAPSNTACCARCNTPPNLKGRYIGELDQNYFTCYAPVIVEPPADLNVTEGMAAELKCRASTSLTSVSWITPNGTVMTHGAYKVRIAVLSDGTLNFTNVTVQDTGMYTCMVSNSVGNTTASATLNVTAATTTPFSYFSTVTVETMEPSQDEARTTDNNVGPTPVVDWETTNVTTSLTPQSTRSTEKTFTIPVTDINSGIPGIDEVMKTTKIIIGCFVAITLMAAVMLVIFYKMRKQHHRQNHHAPTRTVEIINVDDEITGDTPMESHLPMPAIEHEHLNHYNSYKSPFNHTTTVNTINSIHSSVHEPLLIRMNSKDNVQETQI

SEQ ID NO: 6 - protein, 5 aa, Artificial Sequence
  1-15D1 HCDR1
TYVMH

SEQ ID NO: 7 - protein, 17 aa, Artificial Sequence
  1-15D1 HCDR2
YINPYNDNTKYNEKFKG

SEQ ID NO: 8 - protein, 7 aa, Artificial Sequence
  1-15D1 HCDR3
GYDAMDY

SEQ ID NO: 9 - protein, 11 aa, Artificial Sequence
  1-15D1 LCDR1
RTSENIYSHLA

SEQ ID NO: 10 - protein, 7 aa, Artificial Sequence
  1-15D1 LCDR2
SATNLAD

SEQ ID NO: 11 - protein, 9 aa, Artificial Sequence
  1-15D1 LCDR3
QHFWGTPWT

SEQ ID NO: 12 - protein, 17 aa, Artificial Sequence
  1-7F4 HCDR2
YINPYNDKTKYNEKFKG

SEQ ID NO: 13 - protein, 11 aa, Artificial Sequence
  1-7F4 LCDR1
RASENIYSHLA

SEQ ID NO: 14 - protein, 5 aa, Artificial Sequence
  1-10E5 HCDR1
RYTMS

SEQ ID NO: 15 - protein, 17 aa, Artificial Sequence
  1-10E5 HCDR2
TISSGGNSTYYPDSVKG

SEQ ID NO: 16 - protein, 7 aa, Artificial Sequence
  1-10E5 HCDR3
YGYFFDY

SEQ ID NO: 17 - protein, 11 aa, Artificial Sequence
  1-10E5 LCDR1
RASENIYSFLA

SEQ ID NO: 18 - protein, 7 aa, Artificial Sequence
  1-10E5 LCDR2
NAKTLAE

SEQ ID NO: 19 - protein, 9 aa, Artificial Sequence
  1-10E5 LCDR3
QHHYDRPLT

SEQ ID NO: 20 - protein, 4 aa, Artificial Sequence
  14A7 HCDR1
SDFA

SEQ ID NO: 21 - protein, 16 aa, Artificial Sequence
  14A7 HCDR2
YIRFSGSTTYKPTLKS

SEQ ID NO: 22 - protein, 9 aa, Artificial Sequence
  14A7 HCDR3
EDYDGLFDY

SEQ ID NO: 23 - protein, 16 aa, Artificial Sequence
  14A7 LCDR1
RSSQTILHSNGNTYLD

SEQ ID NO: 24 - protein, 7 aa, Artificial Sequence
  14A7 LCDR2
KVSNRFS

SEQ ID NO: 25 - protein, 9 aa, Artificial Sequence
  14A7 LCDR3
FQGSHVPYT

SEQ ID NO: 26 - protein, 116 aa, Artificial Sequence
  The amino acid sequence of 1-15D1 heavy chain variable region
EVQLQQSGPELVKPGASVKMSCKASGYTFTTYVMHWVKQKPGQGLEWIGYINPYNDNTKYNEKFKGKATLTSDKSSSTAYMELSSLTSEDSAVYYCGSGYDAMDYWGQGTSVTVSS

SEQ ID NO: 27 - protein, 107 aa, Artificial Sequence
  The amino acid sequence of 1-15D1 light chain variable region
DIQMAQSPASLSVSVGETVTITCRTSENIYSHLAWYQQKQGKSPQLLVYSATNLADGVPSRFNGSGSGTQYSLKINSLQSEDFGSYYCQHFWGTPWTFGGGTKLEIK

SEQ ID NO: 28 - protein, 116 aa, Artificial Sequence
  The amino acid sequence of 1-7F4 heavy chain variable region
EVQLQQSGPELVKPGASVKMSCKASGYTFTTYVMHWVKQKPGQGLEWIGYINPYNDKTKYNEKFKGKATLTSDKSSSTAYMEVSRLTSEDSAVYYCGSGYDAMDYWGQGTSVTVSS

SEQ ID NO: 29 - protein, 107 aa, Artificial Sequence
  The amino acid sequence of 1-7F4 light chain variable region
DIQMTQSPASLSVSVGETVTITCRASENIYSHLAWYQQKQGKSPQLLIYSATNLADGVPSRFNGSGSGTQYSLKINSLQSEDFGSYYCQHFWGTPWTFGGGTKLEIK

SEQ ID NO: 30 - protein, 116 aa, Artificial Sequence
  The amino acid sequence of 1-10E5 heavy chain variable region
DVKLVESGGGLVKPGGSLKLSCVVSGLTFSRYTMSWVRQTPEKRLEWVATISSGGNSTYYPDSVKGRFTISRDDAKDTLYLQMSSLKSEDTAMYYCTNYGYFFDYWGQGTTLTVSS

SEQ ID NO: 31 - protein, 107 aa, Artificial Sequence
  The amino acid sequence of 1-10E5 light chain variable region
DIQMTQSPASLSASVGETVTITCRASENIYSFLAWYQQKQGKSPQLLVYNAKTLAEGVPSRFSGSGSGTQFSLKINSLQPEDFGSYYCQHHYDRPLTFGAGTKLELK

SEQ ID NO: 32 - protein, 118 aa, Artificial Sequence
  The amino acid sequence of 14A7 heavy chain variable region
DVQLQESGPGLVKPSQSLSLTCTVTGYSITSDFAWNWIRQFPGNKLEWMGYIRFSGSTTYKPTLKSRISITRDTSKNQFFLQLNSVTTEDSATYYCAREDYDGLFDYWGQGTTLTVTS

SEQ ID NO: 33 - protein, 112 aa, Artificial Sequence
  The amino acid sequence of 14A7 light chain variable region
DVLMTQTPLSLPVSLGDHASISCRSSQTILHSNGNTYLDWYLQKPGQSPKLLIYKVSNRFSGVPDRFSGSGSGTDFTLKISRVEAEDLGVYYCFQGSHVPYTFGGGTKLEIK